European Patent Application EP 4 206 230 A1, published July 5, 2023. Title: An humanized antibody to Digoxigenin and use thereof. Applicant: National Cancer Center JP BIO A Inc. Kookmin University Industry Academy Cooperation Foundation. The sequence listing filed with the application follows.

SEQUENCE LISTING (40 sequences)

SEQ ID NO: 1 - protein, 121 aa, Artificial Sequence
  Mus musculus VH-m
QVTLKESGPGILQPSQTLSLTCSLSGFSLTTSGMGVGWIRQSSGKGLEWLANIWWYDTKYYNAALKSRLTISKDTSKNQVFLKIVSVDTADTATYYCGRIHYNGSRFGDYWGQGTTLTVSS

SEQ ID NO: 2 - protein, 122 aa, Artificial Sequence
  Humanized VH-h1
QVTLKESGPTLVKPTQTLTLTCTLSGFSLTTSGMGVGWIRQPPGKALEWVLANIWWYDTKYYNASLKSRLTITKDTSKNQVVLTMTNMDPVDTATYYCGRIHYNGSRFGDYWGQGTLVTVSS

SEQ ID NO: 3 - protein, 121 aa, Artificial Sequence
  Humanized VH-h2
QITLKESGPTLVKPTQTLTLTCTLSGFSLTTSGMGVGWIRQPPGKALEWLANLWWYDTKYYNASLKSRLTITKDTSKNQVVLTMTNMDPVDTATYYCGRLHYNGSRFGDYWGQGTLVTVSS

SEQ ID NO: 4 - protein, 121 aa, Artificial Sequence
  Humanized VH-h3
QVTLQESGPGLVKPSETLSLTCTLSGFSLTTSGMGVGWIRQPPGKGLEWLANIWWYDTKYYNASLKSRVTISKDTSKNQVSLKLSSVTAADTAVYYCGRIHYNGSRFGDYWGQGTLVTVSS

SEQ ID NO: 5 - protein, 121 aa, Artificial Sequence
  Humanized VH-h4
QVQLQESGPGLVKPSETLSLTCTLSGFSLTTSGMGVGWIRQPPGKGLEWIANIWWYDTKYYNASLKSRVTISKDTSKNQVSLKLSSVTAADTAVYYCGRIHYNGSRFGDYWGQGTLVTVSS

SEQ ID NO: 6 - protein, 111 aa, Artificial Sequence
  Mus musculus VL-m
DVVMTQTPLTLSVTFGQPASISCKSSQSLLYTNGKTYLMWLLQRPGQSPKRLIYLVSTLDSGVPGRFSGSGSGTDFTLKISRVEAEDLGVYYCLTIHFPYSFGGGTKLEIK

SEQ ID NO: 7 - protein, 112 aa, Artificial Sequence
  Humanized VL-h1
DVVMTQSPLSLPVTLGQPASISCRSSQSLLYTNGKTYLMWLQQRPGQSPRRLIYLVSTLDSGVPDRFSGSGSGTDFTLKISRVEAEDVGVYYCLQTTHFPYSFGQGTKLEIK

SEQ ID NO: 8 - protein, 112 aa, Artificial Sequence
  Humanized VL-h2
DVVMTQSPLSLPVTLGQPASISCRSSQSLLYTNGKTYLMWLQQRPGQSPRRLIYLVSTWDSGVPDRFSGSGSGTDFTLKISRVEAEDVGVYYCLQTTHFPYSFGQGTKLEIK

SEQ ID NO: 9 - protein, 112 aa, Artificial Sequence
  Humanized VL-h3
DVVMTQSPDSLAVSLGERATINCKSSQSLLYTNGKTYLMWLQQKPGQPPKRLIYLVSTLDSGVPDRFSGSGSGTDFTLTISSLQAEDVAVYYCLQTTHFPYSFGQGTKLEIK

SEQ ID NO: 10 - protein, 112 aa, Artificial Sequence
  Humanized VL-h4
DVVMTQSPDSLAVSLGERATINCKSSQSLLYTNGKTYLMWLQQKPGQPPKRLIYLVSTRDSGVPDRFSGSGSGTDFTLTISSLQAEDVAVYYCLQTTHFPYSFGQGTKLEIK

SEQ ID NO: 11 - DNA, 32 bp, Artificial Sequence
  internal 2'-O-methyl-modified aptamer SQ7-1(8)
  internal 2'-O-methyl-modified aptamers (from 1to 4 and 29 to 32)
  modified_base (1)..(4): 2'-O-methyl-modified bases from 1 to 4
  modified_base (29)..(32): 2'-O-methyl-modified bases from 29 to 32
guuggtatatacttctttagcttggaaccaac

SEQ ID NO: 12 - DNA, 80 bp, Artificial Sequence
  DNA aptamer SQ7
agcagcacagaggtcagatgatgttggtatatacttctttagcttggaaccaactcttgccctatgcgtgctaccgtgaa

SEQ ID NO: 13 - DNA, 32 bp, Artificial Sequence
  DNA aptamer SQ7-1
gttggtatatacttctttagcttggaaccaac

SEQ ID NO: 14 - DNA, 32 bp, Artificial Sequence
  internal 2'-O-methyl-modified aptamer SQ7-1(1)
  internal 2'-O-methyl-modified aptamers (from 1 to 6)
guugguatatacttctttagcttggaaccaac

SEQ ID NO: 15 - DNA, 32 bp, Artificial Sequence
  internal 2'-O-methyl-modified aptamer SQ7-1(2)
  internal 2'-O-methyl-modified aptamers (from 7 to 11)
  modified_base (7)..(11): 2'-O-methyl-modified bases from 7 to 11
gttggtauauacttctttagcttggaaccaac

SEQ ID NO: 16 - DNA, 32 bp, Artificial Sequence
  internal 2'-O-methyl-modified aptamer SQ7-1(3)
  internal 2'-O-methyl-modified aptamers (from 14 to 18)
  modified_base (14)..(18): 2'-O-methyl-modified bases from 14 to 18
gttggtatatactucuuuagcttggaaccaac

SEQ ID NO: 17 - DNA, 32 bp, Artificial Sequence
  internal 2'-O-methyl-modified aptamer SQ7-1(4)
  internal 2'-O-methyl-modified aptamer (from 21 to 26)
  modified_base (21)..(26): 2'-O-methyl-modified bases from 21 to 26
gttggtatatacttctttagcuuggaaccaac

SEQ ID NO: 18 - DNA, 32 bp, Artificial Sequence; identical to SEQ ID NO: 13
  internal 2'-O-methyl-modified aptamer SQ7-1(5)
  internal 2'-O-methyl-modified aptamers (from 27 to 32)
  modified_base (27)..(32): 2'-O-methyl-modified bases from 27 to 32

SEQ ID NO: 19 - DNA, 32 bp, Artificial Sequence
  internal 2'-O-methyl-modified aptamer SQ7-1(6)
  internal 2'-O-methyl-modified aptamers (from 7 to 26)
  modified_base (7)..(26): 2'-O-methyl-modified bases from 7 to 26
gttggtauauacuucuuuagcuuggaaccaac

SEQ ID NO: 20 - DNA, 32 bp, Artificial Sequence; identical to SEQ ID NO: 14
  internal 2'-O-methyl-modified aptamer SQ7-1(1,5)
  internal 2'-O-methyl-modified aptamers (from 1 to 6 and 27 to 32)
  modified_base (1)..(6): 2'-O-methyl-modified bases from 1 to 6
  modified_base (27)..(32): 2'-O-methyl-modified bases from 27 to 32

SEQ ID NO: 21 - DNA, 32 bp, Artificial Sequence; identical to SEQ ID NO: 11
  internal 2'-O-methyl-modified aptamer SQ7-1(7)
  Artificial Sequence
  modified_base (1)..(5): 2'-O-methyl-modified bases from 1 to 5
  modified_base (27)..(32): 2'-O-methyl-modified bases from 27 to 32

SEQ ID NO: 22 - DNA, 32 bp, Artificial Sequence; identical to SEQ ID NO: 11
  internal 2'-O-methyl-modified aptamer SQ7-1(9)
  Artificial Sequence
  modified_base (1)..(3): 2'-O-methyl-modified bases from 1 to 3
  modified_base (30)..(32): 2'-O-methyl-modified bases from 30 to 32

SEQ ID NO: 23 - DNA, 79 bp, Artificial Sequence
  DNA aptamer SQ7a
agcagcacagaggtcagatgatgttggtatatacttctttagcttggaaccaactcttctcctatgcgtgctaccgtga

SEQ ID NO: 24 - DNA, 80 bp, Artificial Sequence
  DNA aptamer SQ7b
agcaacacagaggtcagatgatgttggtatatacttctttagcttggaacccactcttgtcctatgcgtgctaccgtgaa

SEQ ID NO: 25 - DNA, 80 bp, Artificial Sequence
  DNA aptamer SQ1
agcagcacagaggtcagatgcttgggctatctcttattcatgctgttccaccgctctcggcctatgcgtgctaccgtgaa

SEQ ID NO: 26 - DNA, 79 bp, Artificial Sequence
  DNA aptamer SQ2
agcagcacagaggtcagatgaaccgcgatctcatctgtacgctcacccggtcgaagggacctatgcgtgctaccgtgaa

SEQ ID NO: 27 - DNA, 80 bp, Artificial Sequence
  DNA aptamer SQ3
agcagcacagaggtcagatgtgggggcgattacgacccggcgaaattaatagatctgccgcctatgcgtgctaccgtgaa

SEQ ID NO: 28 - DNA, 80 bp, Artificial Sequence
  DNA aptamer SQ4
agcagcacagaggtcagatgagtgtccaacgtcggcgaaattaataggttggaacgaacgcctatgcgtgctaccgtgaa

SEQ ID NO: 29 - DNA, 80 bp, Artificial Sequence
  DNA aptamer SQ5
agcagcacagaggtcagatgtcatggcaaaacgtccctacgctacgattagttaggtcgacctatgcgtgctaccgtgaa

SEQ ID NO: 30 - DNA, 80 bp, Artificial Sequence
  DNA aptamer SQ6
agcagcacagaggtcagatggcttgccacaacgtgcgacgctatgactaattcggcgacccctatgcgtgctaccgtgaa

SEQ ID NO: 31 - DNA, 80 bp, Artificial Sequence
  DNA aptamer SQ8
agcagcacagaggtcagatgcttgggctatttcttattcatgctgttccaccgctctcggcctatgcgtgctaccgtgaa

SEQ ID NO: 32 - DNA, 80 bp, Artificial Sequence
  DNA aptamer SQ9
agcagcacagaggtcagatgattcaactttgaataagtccagtgacttctaacatagtggcctatgcgtgctaccgtgaa

SEQ ID NO: 33 - DNA, 80 bp, Artificial Sequence
  DNA aptamer SQ10
agcagcacagaggtcagatgctcttgaagggatacattgcccttcgatgcttgtctgatccctatgcgtgctaccgtgaa

SEQ ID NO: 34 - DNA, 80 bp, Artificial Sequence
  DNA aptamer SQ11
agcagcacagaggtcagatggtgccaacctgaagtgactgagatatcaaccggtaggcctcctatgcgtgctaccgtgaa

SEQ ID NO: 35 - DNA, 43 bp, Artificial Sequence
  DNA aptamer SQ8-1
cagcacagaggtcagatgcttgggctatttcttattcatgctg

SEQ ID NO: 36 - DNA, 26 bp, Artificial Sequence
  DNA aptamer SQ8-2
cagcacagaggtcagatgcttgggct

SEQ ID NO: 37 - DNA, 32 bp, Artificial Sequence
  DNA aptamer SQ8-3
catgctgttccaccgctctcggcctatgcgtg

SEQ ID NO: 38 - DNA, 28 bp, Artificial Sequence
  DNA aptamer SQ8-4
agcagcacagaggtcagatgcttgggct

SEQ ID NO: 39 - DNA, 23 bp, Artificial Sequence
  DNA aptamer SQ8-5
ctcggcctatgcgtgctaccgtg

SEQ ID NO: 40 - DNA, 30 bp, Artificial Sequence
  DNA aptamer SQ8-6
caccgctctcggcctatgcgtgctaccgtg